European Patent Application EP 4 219 742 A1, published August 2, 2023. Title: DNA impurities in a composition comprising a parvoviral virion. Applicant: uniQure IP B.V. The sequence listing filed with the application follows.

SEQUENCE LISTING (34 sequences)

SEQ ID NO: 1 - DNA, 145 bp, adeno-associated virus 2
  misc_feature 1..145: note = upstream ITR
  source 1..145: mol_type = unassigned DNA
ttggccactccctctctgcgcgctcgctcgctcactgaggccgggcgaccaaaggtcgcccgacgcccgggctttgcccgggcggcctcagtgagcgagcgagcgcgcagagagggagtggccaactccatcactaggggttcct

SEQ ID NO: 2 - DNA, 183 bp, adeno-associated virus 2
  misc_feature 1..183: note = downstream ITR
  source 1..183: mol_type = unassigned DNA
gcgcggtaccccatggaggaacccctagtgatggagttggccactccctctctgcgcgctcgctcgctcactgaggccgcccgggcaaagcccgggcgtcgggcgacctttggtcgcccggcctcagtgagcgagcgagcgcgcagagagggagtggccaagatatcccatggggtaccgcgc

SEQ ID NO: 3 - DNA, 2203 bp, adeno-associated virus 5
  misc_feature 1..2203: note = pDP5
  source 1..2203: mol_type = unassigned DNA
atgtcttttgttgatcaccctccagattggttggaagaagttggtgaaggtcttcgcgagtttttgggccttgaagcgggcccaccgaaaccaaaacccaatcagcagcatcaagatcaagcccgtggtcttgtgctgcctggttataactatctcggacccggaaacggtctcgatcgaggagagcctgtcaacagggcagacgaggtcgcgcgagagcacgacatctcgtacaacgagcagcttgaggcgggagacaacccctacctcaagtacaaccacgcggacgccgagtttcaggagaagctcgccgacgacacatccttcgggggaaacctcggaaaggcagtctttcaggccaagaaaagggttctcgaaccttttggcctggttgaagagggtgctaagacggcccctaccggaaagcggatagacgaccactttccaaaaagaaagaaggctcggaccgaagaggactccaagccttccacctcgtcagacgccgaagctggacccagcggatcccagcagctgcaaatcccagcccaaccagcctcaagtttgggagctgatacaatgtctgcgggaggtggcggcccattgggcgacaataaccaaggtgccgatggagtgggcaatgcctcgggagattggcattgcgattccacgtggatgggggacagagtcgtcaccaagtccacccgaacctgggtgctgcccagctacaacaaccaccagtaccgagagatcaaaagcggctccgtcgacggaagcaacgccaacgcctactttggatacagcaccccctgggggtactttgactttaaccgcttccacagccactggagcccccgagactggcaaagactcatcaacaactactggggcttcagaccccggtccctcagagtcaaaatcttcaacattcaagtcaaagaggtcacggtgcaggactccaccaccaccatcgccaacaacctcacctccaccgtccaagtgtttacggacgacgactaccagctgccctacgtcgtcggcaacgggaccgagggatgcctgccggccttccctccgcaggtctttacgctgccgcagtacggttacgcgacgctgaaccgcgacaacacagaaaatcccaccgagaggagcagcttcttctgcctagagtactttcccagcaagatgctgagaacgggcaacaactttgagtttacctacaactttgaggaggtgcccttccactccagcttcgctcccagtcagaacctgttcaagctggccaacccgctggtggaccagtacttgtaccgcttcgtgagcacaaataacactggcggagtccagttcaacaagaacctggccgggagatacgccaacacctacaaaaactggttcccggggcccatgggccgaacccagggctggaacctgggctccggggtcaaccgcgccagtgtcagcgccttcgccacgaccaataggatggagctcgagggcgcgagttaccaggtgcccccgcagccgaacggcatgaccaacaacctccagggcagcaacacctatgccctggagaacactatgatcttcaacagccagccggcgaacccgggcaccaccgccacgtacctcgagggcaacatgctcatcaccagcgagagcgagacgcagccggtgaaccgcgtggcgtacaacgtcggcgggcagatggccaccaacaaccagagctccaccactgcccccgcgaccggcacgtacaacctccaggaaatcgtgcccggcagcgtgtggatggagagggacgtgtacctccaaggacccatctgggccaagatcccagagacgggggcgcactttcacccctctccggccatgggcggattcggactcaaacacccaccgcccatgatgctcatcaagaacacgcctgtgcccggaaatatcaccagcttctcggacgtgcccgtcagcagcttcatcacccagtacagcaccgggcaggtcaccgtggagatggagtgggagctcaagaaggaaaactccaagaggtggaacccagagatccagtacacaaacaactacaacgacccccagtttgtggactttgccccggacagcaccggggaatacagaaccaccagacctatcggaacccgataccttacccgacccctttaacccattcatgtcgcataccctcaataaa

SEQ ID NO: 4 - DNA, 1876 bp, adeno-associated virus 2
  source 1..1876: mol_type = unassigned DNA
  CDS 11..1876
cgcagccgccatgccggggttttacgagattgtgattaaggtccccagcgaccttgacgagcatctgcccggcatttctgacagctttgtgaactgggtggccgagaaggaatgggagttgccgccagattctgacatggatctgaatctgattgagcaggcacccctgaccgtggccgagaagctgcagcgcgactttctgacggaatggcgccgtgtgagtaaggccccggaggcccttttctttgtgcaatttgagaagggagagagctacttccacatgcacgtgctcgtggaaaccaccggggtgaaatccatggttttgggacgtttcctgagtcagattcgcgaaaaactgattcagagaatttaccgcgggatcgagccgactttgccaaactggttcgcggtcacaaagaccagaaatggcgccggaggcgggaacaaggtggtggatgagtgctacatccccaattacttgctccccaaaacccagcctgagctccagtgggcgtggactaatatggaacagtatttaagcgcctgtttgaatctcacggagcgtaaacggttggtggcgcagcatctgacgcacgtgtcgcagacgcaggagcagaacaaagagaatcagaatcccaattctgatgcgccggtgatcagatcaaaaacttcagccaggtacatggagctggtcgggtggctcgtggacaaggggattacctcggagaagcagtggatccaggaggaccaggcctcatacatctccttcaatgcggcctccaactcgcggtcccaaatcaaggctgccttggacaatgcgggaaagattatgagcctgactaaaaccgcccccgactacctggtgggccagcagcccgtggaggacatttccagcaatcggatttataaaattttggaactaaacgggtacgatccccaatatgcggcttccgtctttctgggatgggccacgaaaaagttcggcaagaggaacaccatctggctgtttgggcctgcaactaccgggaagaccaacatcgcggaggccatagcccacactgtgcccttctacgggtgcgtaaactggaccaatgagaactttcccttcaacgactgtgtcgacaagatggtgatctggtgggaggaggggaagatgaccgccaaggtcgtggagtcggccaaagccattctcggaggaagcaaggtgcgcgtggaccagaaatgcaagtcctcggcccagatagacccgactcccgtgatcgtcacctccaacaccaacatgtgcgccgtgattgacgggaactcaacgaccttcgaacaccagcagccgttgcaagaccggatgttcaaatttgaactcacccgccgtctggatcatgactttgggaaggtcaccaagcaggaagtcaaagactttttccggtgggcaaaggatcacgtggttgaggtggagcatgaattctacgtcaaaaagggtggagccaagaaaagacccgcccccagtgacgcagatataagtgagcccaaacgggtgcgcgagtcagttgcgcagccatcgacgtcagacgcggaagcttcgatcaactacgcagacaggtaccaaaacaaatgttctcgtcacgtgggcatgaatctgatgctgtttccctgcagacaatgcgagagaatgaatcagaattcaaatatctgcttcactcacggacagaaagactgtttagagtgctttcccgtgtcagaatctcaacccgtttctgtcgtcaaaaaggcgtatcagaaactgtgctacattcatcatatcatgggaaaggtgccagacgcttgcactgcctgcgatctggtcaatgtggatttggatgactgcatctttgaacaataa

SEQ ID NO: 5 - protein, 621 aa, adeno-associated virus 2
MPGFYEIVIKVPSDLDEHLPGISDSFVNWVAEKEWELPPDSDMDLNLIEQAPLTVAEKLQRDFLTEWRRVSKAPEALFFVQFEKGESYFHMHVLVETTGVKSMVLGRFLSQIREKLIQRIYRGIEPTLPNWFAVTKTRNGAGGGNKVVDECYIPNYLLPKTQPELQWAWTNMEQYLSACLNLTERKRLVAQHLTHVSQTQEQNKENQNPNSDAPVIRSKTSARYMELVGWLVDKGITSEKQWIQEDQASYISFNAASNSRSQIKAALDNAGKIMSLTKTAPDYLVGQQPVEDISSNRIYKILELNGYDPQYAASVFLGWATKKFGKRNTIWLFGPATTGKTNIAEAIAHTVPFYGCVNWTNENFPFNDCVDKMVIWWEEGKMTAKVVESAKAILGGSKVRVDQKCKSSAQIDPTPVIVTSNTNMCAVIDGNSTTFEHQQPLQDRMFKFELTRRLDHDFGKVTKQEVKDFFRWAKDHVVEVEHEFYVKKGGAKKRPAPSDADISEPKRVRESVAQPSTSDAEASINYADRYQNKCSRHVGMNLMLFPCRQCERMNQNSNICFTHGQKDCLECFPVSESQPVSVVKKAYQKLCYIHHIMGKVPDACTACDLVNVDLDDCIFEQ

SEQ ID NO: 6 - DNA, 1194 bp, synthetic construct
  misc_feature 1..1194: note = AAV2 Rep52 AcMNPV optimized
  misc_feature 1..1194: note = AcMNPV optimized Rep52 coding sequence
  source 1..1194: mol_type = other DNA
atggaattggtcggttggttggtggacaagggtattacctcggagaagcaatggatacaagaagatcaagcctcatacatctcgtttaatgcggcatccaactcgcgtagccaaatcaaagctgccttggacaatgcgggcaagattatgagcctgactaaaaccgcccccgactacctggtgggccagcaacccgtggaagacatttccagcaatcgcatctataagattttggagttaaacggctacgatcctcaatatgcggcttccgtatttttgggctgggcgacgaaaaagtttggcaaaagaaacaccatttggttgtttggacctgcaactacgggaaaaacaaacatagcggaggccatagcccacactgtacctttttatggctgcgttaactggaccaatgagaactttccattcaacgactgtgtcgacaagatggttatttggtgggaggaaggcaaaatgaccgctaaagtcgtggagtcggccaaagcaattttaggaggcagcaaagtgcgcgtagaccagaaatgcaaaagctctgcgcagatagacccgacaccggtgatcgttacaagcaacacgaacatgtgcgccgtgattgacggtaacagtacgacattcgaacaccaacaaccgttgcaagaccgaatgttcaaatttgaattgacgcgccgactggatcatgattttggcaaggtaacaaaacaagaagtcaaagacttctttcgttgggcaaaggatcacgttgttgaagtggaacatgaattttacgtcaaaaaaggtggtgctaagaaaagacccgccccgagtgatgcagatataagtgagcccaaacgagtgagagaatcggttgcgcagccaagcacgtcagatgcggaagcttcgataaactacgcagaccgctaccaaaacaaatgttctcgtcacgtaggcatgaacttaatgttgtttccctgcagacaatgtgagagaatgaatcagaatagtaatatctgtttcactcacggccagaaagactgtttagaatgctttccggtgtcagaatctcaacccgtttctgtcgtaaaaaaggcgtatcaaaaattatgctatattcatcatatcatgggaaaagtgccagacgcttgtactgcctgcgatctggttaatgtggatttggatgactgtatctttgaacaataa

SEQ ID NO: 7 - DNA, 19 bp, synthetic construct
  misc_feature 1..19: note = primer
  misc_feature 1..19: note = pr59
  source 1..19: mol_type = other DNA
aatgggcggtaggcgtgta

SEQ ID NO: 8 - DNA, 22 bp, synthetic construct
  misc_feature 1..22: note = primer
  misc_feature 1..22: note = pr60
  source 1..22: mol_type = other DNA
aggcgatctgacggttcactaa

SEQ ID NO: 9 - DNA, 21 bp, synthetic construct
  misc_feature 1..21: note = primer
  misc_feature 1..21: note = pr180
  source 1..21: mol_type = other DNA
cgaaccgatggctggactatc

SEQ ID NO: 10 - DNA, 23 bp, synthetic construct
  misc_feature 1..23: note = primer
  misc_feature 1..23: note = pr181
  source 1..23: mol_type = other DNA
tgctgctacaagatttggcaagt

SEQ ID NO: 11 - DNA, 20 bp, synthetic construct
  misc_feature 1..20: note = primer
  misc_feature 1..20: note = pr340
  source 1..20: mol_type = other DNA
atacaaccgttggttgcacg

SEQ ID NO: 12 - DNA, 18 bp, synthetic construct
  misc_feature 1..18: note = primer
  misc_feature 1..18: note = pr341
  source 1..18: mol_type = other DNA
cgggacacgccatgtatt

SEQ ID NO: 13 - DNA, 20 bp, synthetic construct
  misc_feature 1..20: note = primer
  misc_feature 1..20: note = pr402
  source 1..20: mol_type = other DNA
gggagtggcggcgttgattt

SEQ ID NO: 14 - DNA, 24 bp, synthetic construct
  misc_feature 1..24: note = primer
  misc_feature 1..24: note = pr403
  source 1..24: mol_type = other DNA
gcacagttcaagcctcacagccta

SEQ ID NO: 15 - DNA, 22 bp, synthetic construct
  misc_feature 1..22: note = primer
  misc_feature 1..22: note = pr404
  source 1..22: mol_type = other DNA
caaacgtggtttcgtgtgccaa

SEQ ID NO: 16 - DNA, 25 bp, synthetic construct
  misc_feature 1..25: note = primer
  misc_feature 1..25: note = pr405
  source 1..25: mol_type = other DNA
gatgcatgacttcacccacacactt

SEQ ID NO: 17 - DNA, 25 bp, synthetic construct
  misc_feature 1..25: note = primer
  misc_feature 1..25: note = pr406
  source 1..25: mol_type = other DNA
acagccattgtaatgagacgcacaa

SEQ ID NO: 18 - DNA, 25 bp, synthetic construct
  misc_feature 1..25: note = primer
  misc_feature 1..25: note = pr407
  source 1..25: mol_type = other DNA
cctagcgcccgatcagcaactatat

SEQ ID NO: 19 - DNA, 25 bp, synthetic construct
  misc_feature 1..25: note = primer
  misc_feature 1..25: note = pr408
  source 1..25: mol_type = other DNA
taccgactctgctgaagaggaggaa

SEQ ID NO: 20 - DNA, 23 bp, synthetic construct
  misc_feature 1..23: note = primer
  misc_feature 1..23: note = pr409
  source 1..23: mol_type = other DNA
tgcgtctggtgcaaactccttta

SEQ ID NO: 21 - DNA, 22 bp, synthetic construct
  misc_feature 1..22: note = primer
  misc_feature 1..22: note = pr410
  source 1..22: mol_type = other DNA
gattcgtcatggccaccacaaa

SEQ ID NO: 22 - DNA, 23 bp, synthetic construct
  misc_feature 1..23: note = primer
  misc_feature 1..23: note = pr411
  source 1..23: mol_type = other DNA
ccaaagcgcccgttgattatttt

SEQ ID NO: 23 - DNA, 23 bp, synthetic construct
  misc_feature 1..23: note = primer
  misc_feature 1..23: note = pr412
  source 1..23: mol_type = other DNA
gcgtacttgcggctgtcgttgta

SEQ ID NO: 24 - DNA, 25 bp, synthetic construct
  misc_feature 1..25: note = primer
  misc_feature 1..25: note = pr413
  source 1..25: mol_type = other DNA
cgaggtcaagttcaaagggcaacat

SEQ ID NO: 25 - DNA, 24 bp, synthetic construct
  misc_feature 1..24: note = primer
  misc_feature 1..24: note = pr426
  source 1..24: mol_type = other DNA
gcatttcgcagctctccttcaatt

SEQ ID NO: 26 - DNA, 23 bp, synthetic construct
  misc_feature 1..23: note = primer
  misc_feature 1..23: note = pr427
  source 1..23: mol_type = other DNA
cttcaagcgagaacgcagcaatt

SEQ ID NO: 27 - DNA, 20 bp, synthetic construct
  misc_feature 1..20: note = primer
  misc_feature 1..20: note = pr428
  source 1..20: mol_type = other DNA
gtggcgtttgccgtggaaaa

SEQ ID NO: 28 - DNA, 23 bp, synthetic construct
  misc_feature 1..23: note = primer
  misc_feature 1..23: note = pr429
  source 1..23: mol_type = other DNA
tgcagctgtgcgttttgaatgaa

SEQ ID NO: 29 - DNA, 22 bp, synthetic construct
  misc_feature 1..22: note = primer
  misc_feature 1..22: note = pr1018
  source 1..22: mol_type = other DNA
ttgttatgtcaatttgtagcgc

SEQ ID NO: 30 - DNA, 22 bp, synthetic construct
  misc_feature 1..22: note = primer
  misc_feature 1..22: note = pr1019
  source 1..22: mol_type = other DNA
tgcataaagacacagtacaacg

SEQ ID NO: 31 - DNA, 26 bp, synthetic construct
  misc_feature 1..26: note = primer
  misc_feature 1..26: note = pr1020
  source 1..26: mol_type = other DNA
gacatagttcgtttgaaaattatccc

SEQ ID NO: 32 - DNA, 23 bp, synthetic construct
  misc_feature 1..23: note = primer
  misc_feature 1..23: note = pr1021
  source 1..23: mol_type = other DNA
aacgatcaagctgttaataaacg

SEQ ID NO: 33 - DNA, 19 bp, synthetic construct
  misc_feature 1..19: note = primer
  misc_feature 1..19: note = pr1024
  source 1..19: mol_type = other DNA
cgcttcggcgtagtttacc

SEQ ID NO: 34 - DNA, 19 bp, synthetic construct
  misc_feature 1..19: note = primer
  misc_feature 1..19: note = pr1025
  source 1..19: mol_type = other DNA
cgctataagcgcgggttac